European Patent Specification EP 3 283 092 B1, published April 29, 2026. Title: Cell-free plant cell culture suspension supernatant with re-youth activity and/or wound healing activity over skin cells. Applicant: PHYTURE BIOTECH, S.L. The sequence listing filed with the application follows.

SEQUENCE LISTING (3 sequences)

SEQ ID NO: 1 - protein, 4 aa, Artificial
  Synthetic peptide derived from phytosulfokine-beta
  ACETYLATION (1)..(1): Acetylated N-terminal tyrosine
  AMIDATION (4)..(4): Amidation of C-terminal threonine
YIYT

SEQ ID NO: 2 - protein, 4 aa, Artificial
  Synthetic peptide derived from phytosulfokine-beta
  SULFATATION (1)..(1): X is a sulphated Tyrosine (Y)
  ACETYLATION (1)..(1): Acetylated N-terminal Tyrosine
  AMIDATION (4)..(4): Amidated C-terminal Threonine
XIYT

SEQ ID NO: 3 - protein, 4 aa, Artificial
  Synthetic peptide derived from phytosulfokine-beta
  ACETYLATION (1)..(1): Acetylated N-terminal Tyrosine
  SULFATATION (3)..(3): X is a sulphated Tyrosine (Y )
  AMIDATION (4)..(4): Amidated C-terminal Threonine
YIXT